European Patent Application EP 4 696 329 A1, published February 18, 2026. Title: ANTI-ROR1 ANTIBODY AND DRUG CONJUGATE THEREOF. Applicant: BioRay Pharmaceutical Co., Ltd. Application WO. The sequence listing filed with the application follows.

SEQUENCE LISTING (88 sequences)

SEQ ID NO: 1 - protein, 117 aa, synthetic construct
QVQLQESGPGLVKPSETLSLTCTVSGFSLTSYGVHWIRQPPGKGLEWLGVIWAGGFTNYNSALKSRLTISKDNSKNQVSLKLSSVTAADTAVYYCARRGSSYSMDYWGQGTLVTVSS

SEQ ID NO: 2 - protein, 106 aa, synthetic construct
EIVLTQSPATLSLSPGERATLSCSASSNVSYIHWYQQKPGQAPRPWIYEISKLASGIPARFSGSGSGTDYTLTISSLEPEDFAVYYCQQWNYPLITFGQGTKLEIK

SEQ ID NO: 3 - protein, 117 aa, synthetic construct
QVQLKESGPGLVAPSQTLSITCTVSGFSLTSYGVHWVRQPPGKGLEWLGVIWAGGFTNYNSALKSRLSISKDNSKSQVLLKMTSLQTDDTAMYYCARRGSSYSMDYWGQGTSVTVSS

SEQ ID NO: 4 - protein, 106 aa, synthetic construct
EIVLSQSPAITAASLGQKVTITCSASSNVSYIHWYQQRSGTSPRPWIYEISKLASGVPVRFSGSGSGTSYSLTISSMEAEDAAIYYCQQWNYPLITFGSGTKLEIQ

SEQ ID NO: 5 - protein, 5 aa, synthetic construct
SYGVH

SEQ ID NO: 6 - protein, 16 aa, synthetic construct
VIWAGGFTNYNSALKS

SEQ ID NO: 7 - protein, 9 aa, synthetic construct
RGSSYSMDY

SEQ ID NO: 8 - protein, 10 aa, synthetic construct
SASSNVSYIH

SEQ ID NO: 9 - protein, 7 aa, synthetic construct
EISKLAS

SEQ ID NO: 10 - protein, 9 aa, synthetic construct
QQWNYPLIT

SEQ ID NO: 11 - protein, 330 aa, synthetic construct
ASTKGPSVFPLAPSSKSTSGGTAALGCLVKDYFPEPVTVSWNSGALTSGVHTFPAVLQSSGLYSLSSVVTVPSSSLGTQTYICNVNHKPSNTKVDKKVEPKSCDKTHTCPPCPAPELLGGPSVFLFPPKPKDTLMISRTPEVTCVVVDVSHEDPEVKFNWYVDGVEVHNAKTKPREEQYNSTYRVVSVLTVLHQDWLNGKEYKCKVSNKALPAPIEKTISKAKGQPREPQVYTLPPSREEMTKNQVSLTCLVKGFYPSDIAVEWESNGQPENNYKTTPPVLDSDGSFFLYSKLTVDKSRWQQGNVFSCSVMHEALHNHYTQKSLSLSPGK

SEQ ID NO: 12 - protein, 107 aa, synthetic construct [sequence omitted]

SEQ ID NO: 13 - protein, 447 aa, synthetic construct
QVQLQESGPGLVKPSETLSLTCTVSGFSLTSYGVHWIRQPPGKGLEWLGVIWAGGFTNYNSALKSRLTISKDNSKNQVSLKLSSVTAADTAVYYCARRGSSYSMDYWGQGTLVTVSSASTKGPSVFPLAPSSKSTSGGTAALGCLVKDYFPEPVTVSWNSGALTSGVHTFPAVLQSSGLYSLSSVVTVPSSSLGTQTYICNVNHKPSNTKVDKKVEPKSCDKTHTCPPCPAPELLGGPSVFLFPPKPKDTLMISRTPEVTCVVVDVSHEDPEVKFNWYVDGVEVHNAKTKPREEQYNSTYRVVSVLTVLHQDWLNGKEYKCKVSNKALPAPIEKTISKAKGQPREPQVYTLPPSREEMTKNQVSLTCLVKGFYPSDIAVEWESNGQPENNYKTTPPVLDSDGSFFLYSKLTVDKSRWQQGNVFSCSVMHEALHNHYTQKSLSLSPGK

SEQ ID NO: 14 - protein, 213 aa, synthetic construct
EIVLTQSPATLSLSPGERATLSCSASSNVSYIHWYQQKPGQAPRPWIYEISKLASGIPARFSGSGSGTDYTLTISSLEPEDFAVYYCQQWNYPLITFGQGTKLEIKRTVAAPSVFIFPPSDEQLKSGTASVVCLLNNFYPREAKVQWKVDNALQSGNSQESVTEQDSKDSTYSLSSTLTLSKADYEKHKVYACEVTHQGLSSPVTKSFNRGEC

SEQ ID NO: 15 - protein, 447 aa, synthetic construct
QVQLKESGPGLVAPSQTLSITCTVSGFSLTSYGVHWVRQPPGKGLEWLGVIWAGGFTNYNSALKSRLSISKDNSKSQVLLKMTSLQTDDTAMYYCARRGSSYSMDYWGQGTSVTVSSASTKGPSVFPLAPSSKSTSGGTAALGCLVKDYFPEPVTVSWNSGALTSGVHTFPAVLQSSGLYSLSSVVTVPSSSLGTQTYICNVNHKPSNTKVDKKVEPKSCDKTHTCPPCPAPELLGGPSVFLFPPKPKDTLMISRTPEVTCVVVDVSHEDPEVKFNWYVDGVEVHNAKTKPREEQYNSTYRVVSVLTVLHQDWLNGKEYKCKVSNKALPAPIEKTISKAKGQPREPQVYTLPPSREEMTKNQVSLTCLVKGFYPSDIAVEWESNGQPENNYKTTPPVLDSDGSFFLYSKLTVDKSRWQQGNVFSCSVMHEALHNHYTQKSLSLSPGK

SEQ ID NO: 16 - protein, 213 aa, synthetic construct
EIVLSQSPAITAASLGQKVTITCSASSNVSYIHWYQQRSGTSPRPWIYEISKLASGVPVRFSGSGSGTSYSLTISSMEAEDAAIYYCQQWNYPLITFGSGTKLEIQRTVAAPSVFIFPPSDEQLKSGTASVVCLLNNFYPREAKVQWKVDNALQSGNSQESVTEQDSKDSTYSLSSTLTLSKADYEKHKVYACEVTHQGLSSPVTKSFNRGEC

SEQ ID NO: 17 - protein, 5 aa, synthetic construct
RYGVH

SEQ ID NO: 18 - protein, 16 aa, synthetic construct
VIWAGGFTNYNSDLKS

SEQ ID NO: 19 - protein, 9 aa, synthetic construct
RGDSYSMKY

SEQ ID NO: 20 - protein, 10 aa, synthetic construct
SASSQVSYIH

SEQ ID NO: 21 - protein, 7 aa, synthetic construct
ETSKLAS

SEQ ID NO: 22 - protein, 117 aa, synthetic construct
QVQLQESGPGLVKPSETLSLTCTVSGFSLTRYGVHWIRQPPGKGLEWLGVIWAGGFTNYNSDLKSRLTISKDNSKNQVSLKLSSVTAADTAVYYCARRGDSYSMKYWGQGTLVTVSS

SEQ ID NO: 23 - protein, 106 aa, synthetic construct
EIVLTQSPATLSLSPGERATLSCSASSQVSYIHWYQQKPGQAPRPWIYETSKLASGIPARFSGSGSGTDYTLTISSLEPEDFAVYYCQQWNYPLITFGQGTKLEIK

SEQ ID NO: 24 - protein, 117 aa, synthetic construct
QVQLQESGPGLVKPSETLSLTCTVSGFSLTRYGVHWIRQPPGKGLEWIGVIWAGGFTNYNSSLKSRVTISKDNSKNQVSLKLSSVTAADTAVYYCARRGDGYSMQYWGQGTLVTVSS

SEQ ID NO: 25 - protein, 106 aa, synthetic construct
EIVLTQSPATLSLSPGERATLSCSASSQVSYIHWYQQKPGQAPRPWIYEISKLASGIPARFSGSGSGTDYTLTISSLEPEDFAVYYCQQWNYPLITFGQGTKLEIK

SEQ ID NO: 26 - protein, 117 aa, synthetic construct
QVQLQESGPGLVKPSETLSLTCTVSGFSLTRYGVHWIRQPPGKGLEWIGVIWAGGFTNYNSTLKSRVTISKDNSKNQVSLKLSSVTAADTAVYYCARRGNQYSMKYWGQGTLVTVSS

SEQ ID NO: 27 - protein, 106 aa, synthetic construct
EIVLTQSPATLSLSPGERATLSCSASSQVSYIHWYQQKPGQAPRPWIYETSKLASGIPARFSGSGSGTDYTLTISSLEPEDFAVYYCQQWNYPLISFGQGTKLEIK

SEQ ID NO: 28 - protein, 117 aa, synthetic construct
QVQLQESGPGLVKPSETLSLTCTVSGFSLTRYGVHWIRQPPGKGLEWIGVIWAGGFTNYNSALKSRVTISKDNSKNQVSLKLSSVTAADTAVYYCARRGNEYSMSYWGQGTLVTVSS

SEQ ID NO: 29 - protein, 117 aa, synthetic construct
QVQLQESGPGLVKPSETLSLTCTVSGFSLTRYGVHWIRQPPGKGLEWLGVIWAGGFTNYNSGLKSRLTISKDNSKNQVSLKLSSVTAADTAVYYCARRGDQYSMGYWGQGTLVTVSS

SEQ ID NO: 30 - protein, 447 aa, synthetic construct
QVQLQESGPGLVKPSETLSLTCTVSGFSLTRYGVHWIRQPPGKGLEWLGVIWAGGFTNYNSDLKSRLTISKDNSKNQVSLKLSSVTAADTAVYYCARRGDSYSMKYWGQGTLVTVSSASTKGPSVFPLAPSSKSTSGGTAALGCLVKDYFPEPVTVSWNSGALTSGVHTFPAVLQSSGLYSLSSVVTVPSSSLGTQTYICNVNHKPSNTKVDKKVEPKSCDKTHTCPPCPAPELLGGPSVFLFPPKPKDTLMISRTPEVTCVVVDVSHEDPEVKFNWYVDGVEVHNAKTKPREEQYNSTYRVVSVLTVLHQDWLNGKEYKCKVSNKALPAPIEKTISKAKGQPREPQVYTLPPSREEMTKNQVSLTCLVKGFYPSDIAVEWESNGQPENNYKTTPPVLDSDGSFFLYSKLTVDKSRWQQGNVFSCSVMHEALHNHYTQKSLSLSPGK

SEQ ID NO: 31 - protein, 213 aa, synthetic construct
EIVLTQSPATLSLSPGERATLSCSASSQVSYIHWYQQKPGQAPRPWIYETSKLASGIPARFSGSGSGTDYTLTISSLEPEDFAVYYCQQWNYPLITFGQGTKLEIKRTVAAPSVFIFPPSDEQLKSGTASVVCLLNNFYPREAKVQWKVDNALQSGNSQESVTEQDSKDSTYSLSSTLTLSKADYEKHKVYACEVTHQGLSSPVTKSFNRGEC

SEQ ID NO: 32 - protein, 16 aa, synthetic construct
VIWAGGFTNYESDLKS

SEQ ID NO: 33 - protein, 16 aa, synthetic construct
VIWAGGFTNYNADLKS

SEQ ID NO: 34 - protein, 16 aa, synthetic construct
VIWAGGFTNYNVDLKS

SEQ ID NO: 35 - protein, 16 aa, synthetic construct
VIWAGGFTNYNTDLKS

SEQ ID NO: 36 - protein, 16 aa, synthetic construct
VIWAGGFTNYNLDLKS

SEQ ID NO: 37 - protein, 16 aa, synthetic construct
VIWAGGFTNYNIDLKS

SEQ ID NO: 38 - protein, 117 aa, synthetic construct
QVQLQESGPGLVKPSETLSLTCTVSGFSLTRYGVHWIRQPPGKGLEWLGVIWAGGFTNYESDLKSRLTISKDNSKNQVSLKLSSVTAADTAVYYCARRGDSYSMKYWGQGTLVTVSS

SEQ ID NO: 39 - protein, 117 aa, synthetic construct
QVQLQESGPGLVKPSETLSLTCTVSGFSLTRYGVHWIRQPPGKGLEWLGVIWAGGFTNYNADLKSRLTISKDNSKNQVSLKLSSVTAADTAVYYCARRGDSYSMKYWGQGTLVTVSS

SEQ ID NO: 40 - protein, 117 aa, synthetic construct
QVQLQESGPGLVKPSETLSLTCTVSGFSLTRYGVHWIRQPPGKGLEWLGVIWAGGFTNYNVDLKSRLTISKDNSKNQVSLKLSSVTAADTAVYYCARRGDSYSMKYWGQGTLVTVSS

SEQ ID NO: 41 - protein, 117 aa, synthetic construct
QVQLQESGPGLVKPSETLSLTCTVSGFSLTRYGVHWIRQPPGKGLEWLGVIWAGGFTNYNTDLKSRLTISKDNSKNQVSLKLSSVTAADTAVYYCARRGDSYSMKYWGQGTLVTVSS

SEQ ID NO: 42 - protein, 117 aa, synthetic construct
QVQLQESGPGLVKPSETLSLTCTVSGFSLTRYGVHWIRQPPGKGLEWLGVIWAGGFTNYNLDLKSRLTISKDNSKNQVSLKLSSVTAADTAVYYCARRGDSYSMKYWGQGTLVTVSS

SEQ ID NO: 43 - protein, 117 aa, synthetic construct
QVQLQESGPGLVKPSETLSLTCTVSGFSLTRYGVHWIRQPPGKGLEWLGVIWAGGFTNYNIDLKSRLTISKDNSKNQVSLKLSSVTAADTAVYYCARRGDSYSMKYWGQGTLVTVSS

SEQ ID NO: 44 - protein, 447 aa, synthetic construct
QVQLQESGPGLVKPSETLSLTCTVSGFSLTRYGVHWIRQPPGKGLEWLGVIWAGGFTNYESDLKSRLTISKDNSKNQVSLKLSSVTAADTAVYYCARRGDSYSMKYWGQGTLVTVSSASTKGPSVFPLAPSSKSTSGGTAALGCLVKDYFPEPVTVSWNSGALTSGVHTFPAVLQSSGLYSLSSVVTVPSSSLGTQTYICNVNHKPSNTKVDKKVEPKSCDKTHTCPPCPAPELLGGPSVFLFPPKPKDTLMISRTPEVTCVVVDVSHEDPEVKFNWYVDGVEVHNAKTKPREEQYNSTYRVVSVLTVLHQDWLNGKEYKCKVSNKALPAPIEKTISKAKGQPREPQVYTLPPSREEMTKNQVSLTCLVKGFYPSDIAVEWESNGQPENNYKTTPPVLDSDGSFFLYSKLTVDKSRWQQGNVFSCSVMHEALHNHYTQKSLSLSPGK

SEQ ID NO: 45 - protein, 5 aa, synthetic construct
SYAMS

SEQ ID NO: 46 - protein, 16 aa, synthetic construct
SISTGASAYFPDSVKG

SEQ ID NO: 47 - protein, 10 aa, synthetic construct
ITTSTWYFDV

SEQ ID NO: 48 - protein, 11 aa, synthetic construct
KASQDINSYLS

SEQ ID NO: 49 - protein, 7 aa, synthetic construct
RANRLVD

SEQ ID NO: 50 - protein, 9 aa, synthetic construct
LQYDEFPYT

SEQ ID NO: 51 - protein, 118 aa, synthetic construct
EVKLVESGGGLVKPGGSLKLSCAASGFTFSSYAMSWVRQTPEKRLEWVASISTGASAYFPDSVKGRFTISRDNARNILYLQMSSLRSEDTAMYYCARITTSTWYFDVWGAGTTVTVSS

SEQ ID NO: 52 - protein, 107 aa, synthetic construct
DIKMTQSPSSMYASLGERVTITCKASQDINSYLSWFQQKPGKSPKTLIYRANRLVDGVPSRFSGSGSGQDYSLTISSLEYEDMGIYYCLQYDEFPYTFGGGTKLEIK

SEQ ID NO: 53 - protein, 118 aa, synthetic construct
EVQLVESGGGLVKPGGSLRLSCAASGFTFSSYAMSWVRQAPGKGLEWVSSISTGASAYFPDSVKGRFTISRDNAKNSLYLQMNSLRAEDTAVYYCARITTSTWYFDVWGQGTTVTVSS

SEQ ID NO: 54 - protein, 118 aa, synthetic construct
EVQLVESGGGLVQPGGSLRLSCAASGFTFSSYAMSWVRQAPGKGLEWVSSISTGASAYFPDSVKGRFTISRDNSKNTLYLQMNSLRAEDTAVYYCARITTSTWYFDVWGQGTTVTVSS

SEQ ID NO: 55 - protein, 118 aa, synthetic construct
EVQLVESGGGLVQPGGSLRLSCAASGFTFSSYAMSWVRQAPGKGLEWVASISTGASAYFPDSVKGRFTISRDNAKNSLYLQMNSLRAEDTAVYYCARITTSTWYFDVWGQGTTVTVSS

SEQ ID NO: 56 - protein, 118 aa, synthetic construct
EVQLVESGGGLVQPGGSLRLSCAASGFTFSSYAMSWVRQAPGKGLEWVSSISTGASAYFPDSVKGRFTISRDNAKNSLYLQMNSLRAEDTAVYYCARITTSTWYFDVWGQGTTVTVSS

SEQ ID NO: 57 - protein, 107 aa, synthetic construct
DIQMTQSPSSLSASVGDRVTITCKASQDINSYLSWFQQKPGKAPKTLIYRANRLVDGVPSRFSGSGSGQDYTLTISSLQPEDMATYYCLQYDEFPYTFGQGTKLEIK

SEQ ID NO: 58 - protein, 107 aa, synthetic construct
DIQMTQSPSSLSASVGDRVTITCKASQDINSYLSWFQQKPGKAPKTLIYRANRLVDGVPSRFSGSGSGQDYTFTISSLQPEDMATYYCLQYDEFPYTFGQGTKLEIK

SEQ ID NO: 59 - protein, 107 aa, synthetic construct
DIQMTQSPSAMSASVGDRVTITCKASQDINSYLSWFQQKPGKVPKTLIYRANRLVDGVPSRFSGSGSGQEYTLTISSLQPEDMATYYCLQYDEFPYTFGQGTKLEIK

SEQ ID NO: 60 - protein, 107 aa, synthetic construct
DIQMTQSPSSLSASVGDRVTITCKASQDINSYLSWFQQKPGKVPKTLIYRANRLVDGVPSRFSGSGSGQDYTLTISSLQPEDMATYYCLQYDEFPYTFGQGTKLEIK

SEQ ID NO: 61 - protein, 5 aa, synthetic construct
SYPMS

SEQ ID NO: 62 - protein, 10 aa, synthetic construct
YTTSTWYFDV

SEQ ID NO: 63 - protein, 11 aa, synthetic construct
KASQDIYSYLS

SEQ ID NO: 64 - protein, 7 aa, synthetic construct
RANRLVR

SEQ ID NO: 65 - protein, 10 aa, synthetic construct
ITTSTWYMDV

SEQ ID NO: 66 - protein, 10 aa, synthetic construct
YTTSTWYHDV

SEQ ID NO: 67 - protein, 11 aa, synthetic construct
KASQDIFSYLS

SEQ ID NO: 68 - protein, 7 aa, synthetic construct
RANRLVS

SEQ ID NO: 69 - protein, 7 aa, synthetic construct
RANRLVG

SEQ ID NO: 70 - protein, 118 aa, synthetic construct
EVQLVESGGGLVQPGGSLRLSCAASGFTFSSYPMSWVRQAPGKGLEWVSSISTGASAYFPDSVKGRFTISRDNAKNSLYLQMNSLRAEDTAVYYCARYTTSTWYFDVWGQGTTVTVSS

SEQ ID NO: 71 - protein, 107 aa, synthetic construct
DIQMTQSPSAMSASVGDRVTITCKASQDIYSYLSWFQQKPGKVPKTLIYRANRLVRGVPSRFSGSGSGQEYTLTISSLQPEDMATYYCLQYDEFPYTFGQGTKLEIK

SEQ ID NO: 72 - protein, 118 aa, synthetic construct
EVQLVESGGGLVQPGGSLRLSCAASGFTFSSYPMSWVRQAPGKGLEWVSSISTGASAYFPDSVKGRFTISRDNAKNSLYLQMNSLRAEDTAVYYCARITTSTWYMDVWGQGTTVTVSS

SEQ ID NO: 73 - protein, 118 aa, synthetic construct
EVQLVESGGGLVQPGGSLRLSCAASGFTFSSYAMSWVRQAPGKGLEWVSSISTGASAYFPDSVKGRFTISRDNAKNSLYLQMNSLRAEDTAVYYCARYTTSTWYHDVWGQGTTVTVSS

SEQ ID NO: 74 - protein, 118 aa, synthetic construct
EVQLVESGGGLVQPGGSLRLSCAASGFTFSSYAMSWVRQAPGKGLEWVSSISTGASAYFPDSVKGRFTISRDNAKNSLYLQMNSLRAEDTAVYYCARITTSTWYMDVWGQGTTVTVSS

SEQ ID NO: 75 - protein, 107 aa, synthetic construct
DIQMTQSPSAMSASVGDRVTITCKASQDIFSYLSWFQQKPGKVPKTLIYRANRLVSGVPSRFSGSGSGQEYTLTISSLQPEDMATYYCLQYDEFPYTFGQGTKLEIK

SEQ ID NO: 76 - protein, 107 aa, synthetic construct
DIQMTQSPSAMSASVGDRVTITCKASQDIYSYLSWFQQKPGKVPKTLIYRANRLVGGVPSRFSGSGSGQEYTLTISSLQPEDMATYYCLQYDEFPYTFGQGTKLEIK

SEQ ID NO: 77 - protein, 448 aa, synthetic construct
EVQLVESGGGLVQPGGSLRLSCAASGFTFSSYPMSWVRQAPGKGLEWVSSISTGASAYFPDSVKGRFTISRDNAKNSLYLQMNSLRAEDTAVYYCARITTSTWYMDVWGQGTTVTVSSASTKGPSVFPLAPSSKSTSGGTAALGCLVKDYFPEPVTVSWNSGALTSGVHTFPAVLQSSGLYSLSSVVTVPSSSLGTQTYICNVNHKPSNTKVDKKVEPKSCDKTHTCPPCPAPELLGGPSVFLFPPKPKDTLMISRTPEVTCVVVDVSHEDPEVKFNWYVDGVEVHNAKTKPREEQYNSTYRVVSVLTVLHQDWLNGKEYKCKVSNKALPAPIEKTISKAKGQPREPQVYTLPPSREEMTKNQVSLTCLVKGFYPSDIAVEWESNGQPENNYKTTPPVLDSDGSFFLYSKLTVDKSRWQQGNVFSCSVMHEALHNHYTQKSLSLSPGK

SEQ ID NO: 78 - protein, 214 aa, synthetic construct
DIQMTQSPSAMSASVGDRVTITCKASQDIYSYLSWFQQKPGKVPKTLIYRANRLVRGVPSRFSGSGSGQEYTLTISSLQPEDMATYYCLQYDEFPYTFGQGTKLEIKRTVAAPSVFIFPPSDEQLKSGTASVVCLLNNFYPREAKVQWKVDNALQSGNSQESVTEQDSKDSTYSLSSTLTLSKADYEKHKVYACEVTHQGLSSPVTKSFNRGEC

SEQ ID NO: 79 - protein, 232 aa, synthetic construct
EPKSCDKTHTCPPCPAPELLGGPSVFLFPPKPKDTLMISRTPEVTCVVVDVSHEDPEVKFNWYVDGVEVHNAKTKPREEQYNSTYRVVSVLTVLHQDWLNGKEYKCKVSNKALPAPIEKTISKAKGQPREPQVYTLPPSREEMTKNQVSLWCLVKGFYPSDIAVEWESNGQPENNYKTTPPVLDSDGSFFLYSKLTVDKSRWQQGNVFSCSVMHEALHNHYTQKSLSLSPGK

SEQ ID NO: 80 - protein, 232 aa, synthetic construct
EPKSCDKTHTCPPCPAPELLGGPSVFLFPPKPKDTLMISRTPEVTCVVVDVSHEDPEVKFNWYVDGVEVHNAKTKPREEQYNSTYRVVSVLTVLHQDWLNGKEYKCKVSNKALPAPIEKTISKAKGQPREPQVYTLPPSREEMTKNQVSLSCAVKGFYPSDIAVEWESNGQPENNYKTTPPVLDSDGSFFLVSKLTVDKSRWQQGNVFSCSVMHEALHNHYTQKSLSLSPGK

SEQ ID NO: 81 - protein, 447 aa, synthetic construct
QVQLQESGPGLVKPSETLSLTCTVSGFSLTRYGVHWIRQPPGKGLEWLGVIWAGGFTNYESDLKSRLTISKDNSKNQVSLKLSSVTAADTAVYYCARRGDSYSMKYWGQGTLVTVSSASTKGPSVFPLAPSSKSTSGGTAALGCLVKDYFPEPVTVSWNSGALTSGVHTFPAVLQSSGLYSLSSVVTVPSSSLGTQTYICNVNHKPSNTKVDKKVEPKSCDKTHTCPPCPAPELLGGPSVFLFPPKPKDTLMISRTPEVTCVVVDVSHEDPEVKFNWYVDGVEVHNAKTKPREEQYNSTYRVVSVLTVLHQDWLNGKEYKCKVSNKALPAPIEKTISKAKGQPREPQVYTLPPSREEMTKNQVSLWCLVKGFYPSDIAVEWESNGQPENNYKTTPPVLDSDGSFFLYSKLTVDKSRWQQGNVFSCSVMHEALHNHYTQKSLSLSPGK

SEQ ID NO: 82 - protein, 213 aa, synthetic construct; identical to SEQ ID NO: 31

SEQ ID NO: 83 - protein, 448 aa, synthetic construct
EVQLVESGGGLVQPGGSLRLSCAASGFTFSSYPMSWVRQAPGKGLEWVSSISTGASAYFPDSVKGRFTISRDNAKNSLYLQMNSLRAEDTAVYYCARITTSTWYMDVWGQGTTVTVSSASTKGPSVFPLAPSSKSTSGGTAALGCLVKDYFPEPVTVSWNSGALTSGVHTFPAVLQSSGLYSLSSVVTVPSSSLGTQTYICNVNHKPSNTKVDKKVEPKSCDKTHTCPPCPAPELLGGPSVFLFPPKPKDTLMISRTPEVTCVVVDVSHEDPEVKFNWYVDGVEVHNAKTKPREEQYNSTYRVVSVLTVLHQDWLNGKEYKCKVSNKALPAPIEKTISKAKGQPREPQVYTLPPSREEMTKNQVSLSCAVKGFYPSDIAVEWESNGQPENNYKTTPPVLDSDGSFFLVSKLTVDKSRWQQGNVFSCSVMHEALHNHYTQKSLSLSPGK

SEQ ID NO: 84 - protein, 214 aa, synthetic construct; identical to SEQ ID NO: 78

SEQ ID NO: 85 - protein, 446 aa, synthetic construct
QVQLQESGPGLVKPSQTLSLTCTVSGYAFTAYNIHWVRQAPGQGLEWMGSFDPYDGGSSYNQKFKDRLTISKDTSKNQVVLTMTNMDPVDTATYYCARGWYYFDYWGHGTLVTVSSASTKGPSVFPLAPSSKSTSGGTAALGCLVKDYFPEPVTVSWNSGALTSGVHTFPAVLQSSGLYSLSSVVTVPSSSLGTQTYICNVNHKPSNTKVDKKVEPKSCDKTHTCPPCPAPELLGGPSVFLFPPKPKDTLMISRTPEVTCVVVDVSHEDPEVKFNWYVDGVEVHNAKTKPREEQYNSTYRVVSVLTVLHQDWLNGKEYKCKVSNKALPAPIEKTISKAKGQPREPQVYTLPPSRDELTKNQVSLTCLVKGFYPSDIAVEWESNGQPENNYKTTPPVLDSDGSFFLYSKLTVDKSRWQQGNVFSCSVMHEALHNHYTQKSLSLSPGK

SEQ ID NO: 86 - protein, 214 aa, synthetic construct
DIVMTQTPLSLPVTPGEPASISCRASKSISKYLAWYQQKPGQAPRLLIYSGSTLQSGIPPRFSGSGYGTDFTLTINNIESEDAAYYFCQQHDESPYTFGEGTKVEIKRTVAAPSVFIFPPSDEQLKSGTASVVCLLNNFYPREAKVQWKVDNALQSGNSQESVTEQDSKDSTYSLSSTLTLSKADYEKHKVYACEVTHQGLSSPVTKSFNRGEC

SEQ ID NO: 87 - protein, 937 aa, Homo sapiens
MHRPRRRGTRPPLLALLAALLLAARGAAAQETELSVSAELVPTSSWNISSELNKDSYLTLDEPMNNITTSLGQTAELHCKVSGNPPPTIRWFKNDAPVVQEPRRLSFRSTIYGSRLRIRNLDTTDTGYFQCVATNGKEVVSSTGVLFVKFGPPPTASPGYSDEYEEDGFCQPYRGIACARFIGNRTVYMESLHMQGEIENQITAAFTMIGTSSHLSDKCSQFAIPSLCHYAFPYCDETSSVPKPRDLCRDECEILENVLCQTEYIFARSNPMILMRLKLPNCEDLPQPESPEAANCIRIGIPMADPINKNHKCYNSTGVDYRGTVSVTKSGRQCQPWNSQYPHTHTFTALRFPELNGGHSYCRNPGNQKEAPWCFTLDENFKSDLCDIPACDSKDSKEKNKMEILYILVPSVAIPLAIALLFFFICVCRNNQKSSSAPVQRQPKHVRGQNVEMSMLNAYKPKSKAKELPLSAVRFMEELGECAFGKIYKGHLYLPGMDHAQLVAIKTLKDYNNPQQWTEFQQEASLMAELHHPNIVCLLGAVTQEQPVCMLFEYINQGDLHEFLIMRSPHSDVGCSSDEDGTVKSSLDHGDFLHIAIQIAAGMEYLSSHFFVHKDLAARNILIGEQLHVKISDLGLSREIYSADYYRVQSKSLLPIRWMPPEAIMYGKFSSDSDIWSFGVVLWEIFSFGLQPYYGFSNQEVIEMVRKRQLLPCSEDCPPRMYSLMTECWNEIPSRRPRFKDIHVRLRSWEGLSSHTSSTTPSGGNATTQTTSLSASPVSNLSNPRYPNYMFPSQGITPQGQIAGFIGPPIPQNQRFIPINGYPIPPGYAAFPAAHYQPTGPPRVIQHCPPPKSRSPSSASGSTSTGHVTSLPSSGSNQEANIPLLPHMSIPNHPGGMGITVFGNKSQKPYKIDSKQASLLGDANIHGHTESMISAEL

SEQ ID NO: 88 - protein, 98 aa, synthetic construct
ASTKGPSVFPLAPSSKSTSGGTAALGCLVKDYFPEPVTVSWNSGALTSGVHTFPAVLQSSGLYSLSSVVTVPSSSLGTQTYICNVNHKPSNTKVDKKV